European Patent Application EP 4 506 365 A1, published February 12, 2025. Title: 抗TIGIT-抗PVRIG双特异性抗体、其药物组合物及用途. Applicant: 普米斯生物技术（珠海）有限公司. The sequence listing filed with the application follows.

SEQUENCE LISTING (50 sequences)

SEQ ID NO: 1 - protein, 122 aa, synthetic construct
QLQLQESGPGLVKPAETLSLTCTVSGGSISSYDHYWTWIRQPPGKGLEWIGTVYYSGSTFHNPSLKSRVTIPVDTSKNQFSLKLSSVTAADTAVYYCARVGPDVSHPPFDYWGQGTLVTVSS

SEQ ID NO: 2 - protein, 107 aa, synthetic construct
DIQMTQSPSSLSASVGDRVTITCRASQSISSYLNWYQQKPGKAPKLLIYAASSLQSGVPSRFSGSGSGTDFTLTISSLQPEDFATYYCQQSYSTPITFGGGTKVEIK

SEQ ID NO: 3 - protein, 126 aa, synthetic construct
QVQLVQSGAEVKKPGASVKVSCKASGYAFTGYYMHWVRQAPGQGLEWMGSIIPFSGEANYAQKFQGRVTMTRDTSISTAYMELSRLRSDDTAVYYCARGPGSLDRLWYYYYGMDVWGQGTTVTVSS

SEQ ID NO: 4 - protein, 108 aa, synthetic construct
EIVLTQSPGTLSLSPGERATLSCRASQSVSSSYLAWYQQKPGQAPRLLIYGASSRATGIPDRFSGSGSGTDFTLTISRLEPEDFAVYYCQQYGSSPITFGGGTKVEIK

SEQ ID NO: 5 - protein, 120 aa, synthetic construct
QVQLVQSGAEVKKPGSSVKVSCKASGGTESVDAISWVRQAPGQGLEWMGDIIPFFDTDYAQKFQGRVTITADESTSTAYMELSSLRSEDTAVYYCAREGGTSWTHFFDLWGRGTLVTVSS

SEQ ID NO: 6 - protein, 10 aa, synthetic construct
GGGGSGGGGS

SEQ ID NO: 7 - protein, 711 aa, synthetic construct
QLQLQESGPGLVKPAETLSLTCTVSGGSISSYDHYWTWIRQPPGKGLEWIGTVYYSGSTFHNPSLKSRVTIPVDTSKNQFSLKLSSVTAADTAVYYCARVGPDVSHPPFDYWGQGTLVTVSSASTKGPSVFPLAPSSKSTSGGTAALGCLVKDYFPEPVTVSWNSGALTSGVHTFPAVLQSSGLYSLSSVVTVPSSSLGTQTYICNVNHKPSNTKVDKKVEPKSCDKTHTCPPCPAPELLGGPSVFLFPPKPKDTLMISRTPEVTCVVVDVSHEDPEVKFNWYVDGVEVHNAKTKPREEQYNSTYRVVSVLTVLHQDWLNGKEYKCKVSNKALPAPIEKTISKAKGQPREPQVYTLPPSREEMTKNQVSLTCLVKGFYPSDIAVEWESNGQPENNYKTTPPVLDSDGSFFLYSKLTVDKSRWQQGNVFSCSVMHEALHNHYTQKSLSLSPGGGGGSGGGGSGQVQLVQSGAEVKKPGSSVKVSCKASGGTESVDAISWVRQAPGQCLEWMGDIIPFFDTDYAQKFQGRVTITADESTSTAYMELSSLRSEDTAVYYCAREGGTSWTHFFDLWGRGTLVTVSSGGGGSGGGGSGGGGSGGGGSGEIVLTQSPGTLSLSPGERATLSCRASQSVSSSYLAWYQQKPGQAPRLLIYGASSRATGIPDRFSGSGSGTDFTLTISRLEPEDFAVYYCQQYGSSPITFGCGTKVEIK

SEQ ID NO: 8 - protein, 214 aa, synthetic construct
DIQMTQSPSSLSASVGDRVTITCRASQSISSYLNWYQQKPGKAPKLLIYAASSLQSGVPSRFSGSGSGTDFTLTISSLQPEDFATYYCQQSYSTPITFGGGTKVEIKRTVAAPSVFIFPPSDEQLKSGTASVVCLLNNFYPREAKVQWKVDNALQSGNSQESVTEQDSKDSTYSLSSTLTLSKADYEKHKVYACEVTHQGLSSPVTKSFNRGEC

SEQ ID NO: 9 - protein, 710 aa, synthetic construct
QVQLVQSGAEVKKPGSSVKVSCKASGGTESVDAISWVRQAPGQGLEWMGDIIPFFDTDYAQKFQGRVTITADESTSTAYMELSSLRSEDTAVYYCAREGGTSWTHFFDLWGRGTLVTVSSASTKGPSVFPLAPSSKSTSGGTAALGCLVKDYFPEPVTVSWNSGALTSGVHTFPAVLQSSGLYSLSSVVTVPSSSLGTQTYICNVNHKPSNTKVDKKVEPKSCDKTHTCPPCPAPELLGGPSVFLFPPKPKDTLMISRTPEVTCVVVDVSHEDPEVKFNWYVDGVEVHNAKTKPREEQYNSTYRVVSVLTVLHQDWLNGKEYKCKVSNKALPAPIEKTISKAKGQPREPQVYTLPPSREEMTKNQVSLTCLVKGFYPSDIAVEWESNGQPENNYKTTPPVLDSDGSFFLYSKLTVDKSRWQQGNVFSCSVMHEALHNHYTQKSLSLSPGGGGGSGGGGSGQLQLQESGPGLVKPAETLSLTCTVSGGSISSYDHYWTWIRQPPGKCLEWIGTVYYSGSTFHNPSLKSRVTIPVDTSKNQFSLKLSSVTAADTAVYYCARVGPDVSHPPFDYWGQGTLVTVSSGGGGSGGGGSGGGGSGGGGSGDIQMTQSPSSLSASVGDRVTITCRASQSISSYLNWYQQKPGKAPKLLIYAASSLQSGVPSRFSGSGSGTDFTLTISSLQPEDFATYYCQQSYSTPITFGCGTKVEIK

SEQ ID NO: 10 - protein, 215 aa, synthetic construct
EIVLTQSPGTLSLSPGERATLSCRASQSVSSSYLAWYQQKPGQAPRLLIYGASSRATGIPDRFSGSGSGTDFTLTISRLEPEDFAVYYCQQYGSSPITFGGGTKVEIKRTVAAPSVFIFPPSDEQLKSGTASVVCLLNNFYPREAKVQWKVDNALQSGNSQESVTEQDSKDSTYSLSSTLTLSKADYEKHKVYACEVTHQGLSSPVTKSFNRGEC

SEQ ID NO: 11 - protein, 455 aa, synthetic construct
QVQLVQSGAEVKKPGASVKVSCKASGYAFTGYYMHWVRQAPGQGLEWMGSIIPFSGEANYAQKFQGRVTMTRDTSISTAYMELSRLRSDDTAVYYCARGPGSLDRLWYYYYGMDVWGQGTTVTVSSASTKGPSVFPLAPSSKSTSGGTAALGCLVKDYFPEPVTVSWNSGALTSGVHTFPAVLQSSGLYSLSSVVTVPSSSLGTQTYICNVNHKPSNTKVDKKVEPKSCDKTHTCPPCPAPELLGGPSVFLFPPKPKDTLMISRTPEVTCVVVDVSHEDPEVKFNWYVDGVEVHNAKTKPREEQYNSTYRVVSVLTVLHQDWLNGKEYKCKVSNKALPAPIEKTISKAKGQPREPQVYTLPPCRDELTKNQVSLWCLVKGFYPSDIAVEWESNGQPENNYKTTPPVLDSDGSFFLYSKLTVDKSRWQQGNVFSCSVMHEALHNHYTQKSLSLSPG

SEQ ID NO: 12 - protein, 449 aa, synthetic construct
QVQLVQSGAEVKKPGSSVKVSCKASGGTESVDAISWVRQAPGQGLEWMGDIIPFFDTDYAQKFQGRVTITADESTSTAYMELSSLRSEDTAVYYCAREGGTSWTHFFDLWGRGTLVTVSSASTKGPSVFPLAPSSKSTSGGTAALGCLVKDYFPEPVTVSWNSGALTSGVHTFPAVLQSSGLYSLSSVVTVPSSSLGTQTYICNVNHKPSNTKVDKKVEPKSCDKTHTCPPCPAPELLGGPSVFLFPPKPKDTLMISRTPEVTCVVVDVSHEDPEVKFNWYVDGVEVHNAKTKPREEQYNSTYRVVSVLTVLHQDWLNGKEYKCKVSNKALPAPIEKTISKAKGQPREPQVCTLPPSRDELTKNQVSLSCAVKGFYPSDIAVEWESNGQPENNYKTTPPVLDSDGSFFLVSKLTVDKSRWQQGNVFSCSVMHEALHNHYTQKSLSLSPG

SEQ ID NO: 13 - protein, 11 aa, synthetic construct
GSISSYDHYWT

SEQ ID NO: 14 - protein, 16 aa, synthetic construct
TVYYSGSTFHNPSLKS

SEQ ID NO: 15 - protein, 14 aa, synthetic construct
ARVGPDVSHPPFDY

SEQ ID NO: 16 - protein, 11 aa, synthetic construct
RASQSISSYLN

SEQ ID NO: 17 - protein, 7 aa, synthetic construct
AASSLQS

SEQ ID NO: 18 - protein, 9 aa, synthetic construct
QQSYSTPIT

SEQ ID NO: 19 - protein, 9 aa, synthetic construct
YAFTGYYMH

SEQ ID NO: 20 - protein, 17 aa, synthetic construct
SIIPFSGEANYAQKFQG

SEQ ID NO: 21 - protein, 19 aa, synthetic construct
ARGPGSLDRLWYYYYGMDV

SEQ ID NO: 22 - protein, 12 aa, synthetic construct
RASQSVSSSYLA

SEQ ID NO: 23 - protein, 7 aa, synthetic construct
GASSRAT

SEQ ID NO: 24 - protein, 9 aa, synthetic construct
QQYGSSPIT

SEQ ID NO: 25 - protein, 9 aa, synthetic construct
GTESVDAIS

SEQ ID NO: 26 - protein, 16 aa, synthetic construct
DIIPFFDTDYAQKFQG

SEQ ID NO: 27 - protein, 14 aa, synthetic construct
AREGGTSWTHFFDL

SEQ ID NO: 28 - protein, 171 aa, synthetic construct
MRTEAQVPALQPPEPGLEGAMGHRTLVLPWVLLTLCVTAGTPEVWVQVRMEATELSSFTIRCGFLGSGSISLVTVSWGGPNGAGGTTLAVLHPERGIRQWAPARQARWETQSSISLILEGSGASSPCANTTFCCKFASFPEGSWEACGSLPPSSDPGLSAPPTPAPILRAD

SEQ ID NO: 29 - protein, 171 aa, synthetic construct
MRTEAQVLALQSPEPGLEGAMGRRTLALPWVLLTLCVTAGTPEVWVQVQMEATELSSFTVHCGFLGPGSISLVTVSWGGPDGAGGTKLAVLHPELGTRQWAPARQARWETQSSISLALEDSGASSPFANTTFCCKFASFPEGSWESCGSLPPSSDPGLSAPPTPVPILRAD

SEQ ID NO: 30 - protein, 131 aa, synthetic construct
SPEVWVQVQMEATNLSSFSVHCGVLGYSLISLVTVSCEGFVDAGRTKLAVLHPEFGTQQWAPARQAHWETPNSVSVTLTMGQSKARSSLANTTFCCEFVTFPHGSRVACRDLHRSDPGLSAPTPALNLQAD

SEQ ID NO: 31 - protein, 120 aa, synthetic construct
MMTGTIETTGNISAEKGGSIILQCHLSSTTAQVTQVNWEQQDQLLAICNADLGWHISPSFKDRVAPGPGLGLTLQSLTVNDTGEYFCIYHTYPDGTYTGRIFLEVLESSVAEHGARFQIP

SEQ ID NO: 32 - protein, 121 aa, synthetic construct
MMTGTIETTGNISAKKGGSVILQCHLSSTMAQVTQVNWEQHDHSLLAIRNAELGWHIYPAFKDRVAPGPGLGLTLQSLTMNDTGEYFCTYHTYPDGTYRGRIFLEVLESSVAEHSARFQIP

SEQ ID NO: 33 - protein, 120 aa, synthetic construct
TIDTKRNISAEEGGSVILQCHFSSDTAEVTQVDWKQQDQLLAIYSVDLGWHVASVFSDRVVPGPSLGLTFQSLTMNDTGEYFCTYHTYPGGIYKGRIFLKVQESSDDRNGLAQFQTAPLG

SEQ ID NO: 34 - protein, 120 aa, synthetic construct
QVQLVQSGAEVKKPGASVKVSCKASGYTFTEYYIYWVRQAPGQGLEWIGGINPSNGGTNFNEKFKPRVTMTVDTSTSTAYMELSSLRSEDTAVYYCTVRDFRFDKGFKYWGQGTLVTVSS

SEQ ID NO: 35 - protein, 111 aa, synthetic construct
EIVLTQSPATLSLSPGERATLSCRASKSVSTSGLNYVHWYQRKPGQAPRLLIYLGSYLDSGVPARFSGSGSGTDFTLTISSLEPEDFAVYYCQQSWELPLTFGGGTKVEIK

SEQ ID NO: 36 - protein, 9 aa, synthetic construct
YTFTEYYIY

SEQ ID NO: 37 - protein, 17 aa, synthetic construct
GINPSNGGTNFNEKFKP

SEQ ID NO: 38 - protein, 13 aa, synthetic construct
TVRDFRFDKGFKY

SEQ ID NO: 39 - protein, 15 aa, synthetic construct
RASKSVSTSGLNYVH

SEQ ID NO: 40 - protein, 7 aa, synthetic construct
LGSYLDS

SEQ ID NO: 41 - protein, 9 aa, synthetic construct
QQSWELPLT

SEQ ID NO: 42 - protein, 329 aa, synthetic construct
ASTKGPSVFPLAPSSKSTSGGTAALGCLVKDYFPEPVTVSWNSGALTSGVHTFPAVLQSSGLYSLSSVVTVPSSSLGTQTYICNVNHKPSNTKVDKKVEPKSCDKTHTCPPCPAPEAAGGPSVFLFPPKPKDTLMISRTPEVTCVVVDVSHEDPEVKFNWYVDGVEVHNAKTKPREEQYNSTYRVVSVLTVLHQDWLNGKEYKCKVSNKALPAPIEKTISKAKGQPREPQVYTLPPSRDELTKNQVSLTCLVKGFYPSDIAVEWESNGQPENNYKTTPPVLDSDGSFFLYSKLTVDKSRWQQGNVFSCSVMHEALHNHYTQKSLSLSPG

SEQ ID NO: 43 - protein, 107 aa, synthetic construct [sequence omitted]

SEQ ID NO: 44 - protein, 11 aa, synthetic construct
GGGGSGGGGSG

SEQ ID NO: 45 - protein, 21 aa, synthetic construct
GGGGSGGGGSGGGGSGGGGSG

SEQ ID NO: 46 - protein, 20 aa, synthetic construct
GGGGSGGGGSGGGGSGGGGS

SEQ ID NO: 47 - protein, 122 aa, synthetic construct
QLQLQESGPGLVKPAETLSLTCTVSGGSISSYDHYWTWIRQPPGKCLEWIGTVYYSGSTFHNPSLKSRVTIPVDTSKNQFSLKLSSVTAADTAVYYCARVGPDVSHPPFDYWGQGTLVTVSS

SEQ ID NO: 48 - protein, 107 aa, synthetic construct
DIQMTQSPSSLSASVGDRVTITCRASQSISSYLNWYQQKPGKAPKLLIYAASSLQSGVPSRFSGSGSGTDFTLTISSLQPEDFATYYCQQSYSTPITFGCGTKVEIK

SEQ ID NO: 49 - protein, 120 aa, synthetic construct
QVQLVQSGAEVKKPGSSVKVSCKASGGTESVDAISWVRQAPGQCLEWMGDIIPFFDTDYAQKFQGRVTITADESTSTAYMELSSLRSEDTAVYYCAREGGTSWTHFFDLWGRGTLVTVSS

SEQ ID NO: 50 - protein, 108 aa, synthetic construct
EIVLTQSPGTLSLSPGERATLSCRASQSVSSSYLAWYQQKPGQAPRLLIYGASSRATGIPDRFSGSGSGTDFTLTISRLEPEDFAVYYCQQYGSSPITFGCGTKVEIK